European Patent Application EP 4 286 011 A2, published December 6, 2023. Title: FCRN antibodies and methods of use thereof. Applicant: Momenta Pharmaceuticals, Inc. The sequence listing filed with the application follows.

SEQUENCE LISTING (24 sequences)

SEQ ID NO: 1 - protein, 14 aa, synthetic construct
  REGION 1..14: note = Synthetic construct
TGTGSDVGSYNLVS

SEQ ID NO: 2 - protein, 7 aa, synthetic construct
  REGION 1..7: note = Synthetic construct
GDSERPS

SEQ ID NO: 3 - protein, 10 aa, synthetic construct
  REGION 1..10: note = Synthetic construct
SSYAGSGIYV

SEQ ID NO: 4 - protein, 5 aa, synthetic construct
  REGION 1..5: note = Synthetic construct
TYAMG

SEQ ID NO: 5 - protein, 5 aa, synthetic construct
  REGION 1..5: note = Synthetic construct
DYAMG

SEQ ID NO: 6 - protein, 5 aa, synthetic construct
  REGION 1..5: note = Synthetic construct
NYAMG

SEQ ID NO: 7 - protein, 14 aa, synthetic construct
  REGION 1..14: note = Synthetic construct
SIGSSGAQTRYADS

SEQ ID NO: 8 - protein, 14 aa, synthetic construct
  REGION 1..14: note = Synthetic construct
SIGASGSQTRYADS

SEQ ID NO: 9 - protein, 14 aa, synthetic construct
  REGION 1..14: note = Synthetic construct
SIGASGAQTRYADS

SEQ ID NO: 10 - protein, 14 aa, synthetic construct
  REGION 1..14: note = Synthetic construct
SIGASGGQTRYADS

SEQ ID NO: 11 - protein, 7 aa, synthetic construct
  REGION 1..7: note = Synthetic construct
LAIGDSY

SEQ ID NO: 12 - protein, 14 aa, synthetic construct
  REGION 1..14: note = Synthetic construct
  SITE 1: note = MISC_FEATURE - Xaa is a polar or hydrophobic amino acid, e.g. Thr, Ala, Ser, or Ile
  SITE 12: note = MISC_FEATURE - Xaa is a hydrophobic amino acid, e.g. Leu or Ile
XGTGSDVGSYNXVS

SEQ ID NO: 13 - protein, 7 aa, synthetic construct
  REGION 1..7: note = Synthetic construct
  SITE 3: note = MISC_FEATURE - Xaa is a polar amino acid, e.g. Ser, Asn, or Thr
  SITE 4: note = MISC_FEATURE - Xaa is a polar or acidic amino acid, e.g. Gln, Glu, or Asn
GDXXRPS

SEQ ID NO: 14 - protein, 10 aa, synthetic construct
  REGION 1..10: note = Synthetic construct
  SITE 1: note = MISC_FEATURE - Xaa is a polar or hydrophobic amino acid, e.g. Cys, Ser, Ile, or Tyr
  SITE 4: note = MISC_FEATURE - Xaa is a hydrophobic amino acid, e.g. Ala or Val
XSYXGSGIYV

SEQ ID NO: 15 - protein, 5 aa, synthetic construct
  REGION 1..5: note = Synthetic Construct
  SITE 1: note = MISC_FEATURE - Xaa is a polar or acidic amino acid, e.g. Glu, Thr, Asp, or Asn
XYAMG

SEQ ID NO: 16 - protein, 14 aa, synthetic construct
  REGION 1..14: note = Synthetic Construct
  SITE 4: note = MISC_FEATURE - Xaa is a polar or hydrophobic amino acid, e.g. Ser or Ala
  SITE 7: note = MISC_FEATURE - Xaa is Gly, Ser, or Ala
  SITE 10: note = MISC_FEATURE - Xaa is a basic amino acid, e.g. Gly, Ser, or Ala
SIGXSGXQTXYADS

SEQ ID NO: 17 - protein, 7 aa, synthetic construct
  REGION 1..7: note = Synthetic Construct
  SITE 3: note = MISC_FEATURE - Xaa is a hydrophobic or basic amino acid, e.g. Ile, Leu, or His
  SITE 4: note = MISC_FEATURE - Xaa is Gly, Ser, Asp, Gln, or His
LAXXDSY

SEQ ID NO: 18 - protein, 14 aa, synthetic construct
  REGION 1..14: note = Synthetic Construct
  SITE 4: note = MISC_FEATURE - Xaa is a polar or hydrophobic amino acid, e.g. Ser or Ala
  SITE 7: note = MISC_FEATURE - Xaa is Glu, Ser, or Ala
SIGXSGXQTRYADS

SEQ ID NO: 19 - protein, 216 aa, synthetic construct
  REGION 1..216: note = Synthetic Construct
QSALTQPASVSGSPGQSITISCTGTGSDVGSYNLVSWYQQHPGKAPKLMIYGDSERPSGVSNRFSGSKSGNTASLTISGLQAEDEADYYCSSYAGSGIYVFGTGTKVTVLGQPKAAPSVTLFPPSSEELQANKATLVCLISDFYPGAVTVAWKADSSPVKAGVETTTPSKQSNNKYAASSYLSLTPEQWKSHKSYSCQVTHEGSTVEKTVAPTECS

SEQ ID NO: 20 - protein, 445 aa, synthetic construct
  REGION 1..445: note = Synthetic Construct
EVQLLESGGGLVQPGGSLRLSCAASGFTFSTYAMGWVRQAPGKGLEWVSSIGSSGAQTRYADSVKGRFTISRDNSKNTLYLQMNSLRAEDTAVYYCARLAIGDSYWGQGTMVTVSSASTKGPSVFPLAPSSKSTSGGTAALGCLVKDYFPEPVTVSWNSGALTSGVHTFPAVLQSSGLYSLSSVVTVPSSSLGTQTYICNVNHKPSNTKVDKKVEPKSCDKTHTCPPCPAPELLGGPSVFLFPPKPKDTLMISRTPEVTCVVVDVSHEDPEVKFNWYVDGVEVHNAKTKPREEQYASTYRVVSVLTVLHQDWLNGKEYKCKVSNKALPAPIEKTISKAKGQPREPQVYTLPPSRDELTKNQVSLTCLVKGFYPSDIAVEWESNGQPENNYKTTPPVLDSDGSFFLYSKLTVDKSRWQQGNVFSCSVMHEALHNHYTQKSLSLSPG

SEQ ID NO: 21 - protein, 445 aa, synthetic construct
  REGION 1..445: note = Synthetic Construct
EVQLLESGGGLVQPGGSLRLSCAASGFTFSDYAMGWVRQAPGKGLEWVSSIGASGSQTRYADSVKGRFTISRDNSKNTLYLQMNSLRAEDTAVYYCARLAIGDSYWGQGTMVTVSSASTKGPSVFPLAPSSKSTSGGTAALGCLVKDYFPEPVTVSWNSGALTSGVHTFPAVLQSSGLYSLSSVVTVPSSSLGTQTYICNVNHKPSNTKVDKKVEPKSCDKTHTCPPCPAPELLGGPSVFLFPPKPKDTLMISRTPEVTCVVVDVSHEDPEVKFNWYVDGVEVHNAKTKPREEQYASTYRVVSVLTVLHQDWLNGKEYKCKVSNKALPAPIEKTISKAKGQPREPQVYTLPPSRDELTKNQVSLTCLVKGFYPSDIAVEWESNGQPENNYKTTPPVLDSDGSFFLYSKLTVDKSRWQQGNVFSCSVMHEALHNHYTQKSLSLSPG

SEQ ID NO: 22 - protein, 445 aa, synthetic construct
  REGION 1..445: note = Synthetic Construct
EVQLLESGGGLVQPGGSLRLSCAASGFTFSNYAMGWVRQAPGKGLEWVSSIGASGAQTRYADSVKGRFTISRDNSKNTLYLQMNSLRAEDTAVYYCARLAIGDSYWGQGTMVTVSSASTKGPSVFPLAPSSKSTSGGTAALGCLVKDYFPEPVTVSWNSGALTSGVHTFPAVLQSSGLYSLSSVVTVPSSSLGTQTYICNVNHKPSNTKVDKKVEPKSCDKTHTCPPCPAPELLGGPSVFLFPPKPKDTLMISRTPEVTCVVVDVSHEDPEVKFNWYVDGVEVHNAKTKPREEQYASTYRVVSVLTVLHQDWLNGKEYKCKVSNKALPAPIEKTISKAKGQPREPQVYTLPPSREEMTKNQVSLTCLVKGFYPSDIAVEWESNGQPENNYKTTPPVLDSDGSFFLYSKLTVDKSRWQQGNVFSCSVMHEALHNHYTQKSLSLSPG

SEQ ID NO: 23 - protein, 445 aa, synthetic construct
  REGION 1..445: note = Synthetic Construct
EVQLLESGGGLVQPGGSLRLSCAASGFTFSTYAMGWVRQAPGKGLEWVSSIGASGGQTRYADSVKGRFTISRDNSKNTLYLQMNSLRAEDTAVYYCARLAIGDSYWGQGTMVTVSSASTKGPSVFPLAPSSKSTSGGTAALGCLVKDYFPEPVTVSWNSGALTSGVHTFPAVLQSSGLYSLSSVVTVPSSSLGTQTYICNVNHKPSNTKVDKKVEPKSCDKTHTCPPCPAPELLGGPSVFLFPPKPKDTLMISRTPEVTCVVVDVSHEDPEVKFNWYVDGVEVHNAKTKPREEQYASTYRVVSVLTVLHQDWLNGKEYKCKVSNKALPAPIEKTISKAKGQPREPQVYTLPPSREEMTKNQVSLTCLVKGFYPSDIAVEWESNGQPENNYKTTPPVLDSDGSFFLYSKLTVDKSRWQQGNVFSCSVMHEALHNHYTQKSLSLSPG

SEQ ID NO: 24 - protein, 445 aa, synthetic construct
  REGION 1..445: note = Synthetic Construct
EVQLLESGGGLVQPGGSLRLSCAASGFTFSTYAMGWVRQAPGKGLEWVSSIGASGSQTRYADSVKGRFTISRDNSKNTLYLQMNSLRAEDTAVYYCARLAIGDSYWGQGTMVTVSSASTKGPSVFPLAPSSKSTSGGTAALGCLVKDYFPEPVTVSWNSGALTSGVHTFPAVLQSSGLYSLSSVVTVPSSSLGTQTYICNVNHKPSNTKVDKKVEPKSCDKTHTCPPCPAPELLGGPSVFLFPPKPKDTLMISRTPEVTCVVVDVSHEDPEVKFNWYVDGVEVHNAKTKPREEQYASTYRVVSVLTVLHQDWLNGKEYKCKVSNKALPAPIEKTISKAKGQPREPQVYTLPPSREEMTKNQVSLTCLVKGFYPSDIAVEWESNGQPENNYKTTPPVLDSDGSFFLYSKLTVDKSRWQQGNVFSCSVMHEALHNHYTQKSLSLSPG